European Patent Application EP 4 516 307 A1, published March 5, 2025. Title: 治疗心血管和肾脏疾病的中药组合物及其制备方法. Applicant: 北京博奥晶方生物科技有限公司. The sequence listing filed with the application follows.

SEQUENCE LISTING (8 sequences)

SEQ ID NO: 1 - DNA, 20 bp, synthetic construct
  source 1..20: mol_type = other DNA
tggaaacgtccgggttacag

SEQ ID NO: 2 - DNA, 20 bp, synthetic construct
  source 1..20: mol_type = other DNA
ctgatccggtccatcttcct

SEQ ID NO: 3 - DNA, 21 bp, synthetic construct
  source 1..21: mol_type = other DNA
gagggccaagacgaagacatc

SEQ ID NO: 4 - DNA, 21 bp, synthetic construct
  source 1..21: mol_type = other DNA
cagatcacgtcatcgcacaac

SEQ ID NO: 5 - DNA, 20 bp, synthetic construct
  source 1..20: mol_type = other DNA
taccctgcgtctgcatttcc

SEQ ID NO: 6 - DNA, 21 bp, synthetic construct
  source 1..21: mol_type = other DNA
gctcgttgtagatggagacca

SEQ ID NO: 7 - DNA, 21 bp, synthetic construct
  source 1..21: mol_type = other DNA
agtggacttttcagaggtgga

SEQ ID NO: 8 - DNA, 21 bp, synthetic construct
  source 1..21: mol_type = other DNA
gccgttgaagtagagggcatt